European Patent Application EP 4 129 301 A1, published February 8, 2023. Title: Compuestos para la profilaxis y/o el tratamiento del síndrome de dificultad respiratoria aguda. Applicant: SERVICIO ANDALUZ DE SALUD. The sequence listing filed with the application follows.

SEQUENCE LISTING (2 sequences)

SEQ ID NO: 1 - protein, 427 aa, Homo sapiens
MEAMAASTSLPDPGDFDRNVPRICGVCGDRATGFHFNAMTCEGCKGFFRRSMKRKALFTCPFNGDCRITKDNRRHCQACRLKRCVDIGMMKEFILTDEEVQRKREMILKRKEEEALKDSLRPKLSEEQQRIIAILLDAHHKTYDPTYSDFCQFRPPVRVNDGGGSHPSRPNSRHTPSFSGDSSSSCSDHCITSSDMMDSSSFSNLDLSEEDSDDPSVTLELSQLSMLPHLADLVSYSIQKVIGFAKMIPGFRDLTSEDQIVLLKSSAIEVIMLRSNESFTMDDMSWTCGNQDYKYRVSDVTKAGHSLELIEPLIKFQVGLKKLNLHEEEHVLLMAICIVSPDRPGVQDAALIEAIQDRLSNTLQTYIRCRHPPPGSHLLYAKMIQKLADLRSLNEEHSKQYRCLSFQPECSMKLTPLVLEVFGNEIS

SEQ ID NO: 2 - DNA, 4535 bp, Homo sapiens
gggagcgcggaacagcttgtccacccgccggccggaccagggatggaggcaatggcggccagcacttccctgcctgaccctggagactttgaccggaacgtgccccggatctgtggggtgtgtggagaccgagccactggctttcacttcaatgctatgacctgtgaaggctgcaaaggcttcttcaggcgaagcatgaagcggaaggcactattcacctgccccttcaacggggactgccgcatcaccaaggacaaccgacgccactgccaggcctgccggctcaaacgctgtgtggacatcggcatgatgaaggagttcattctgacagatgaggaagtgcagaggaagcgggagatgatcctgaagcggaaggaggaggaggccttgaaggacagtctgcggcccaagctgtctgaggagcagcagcgcatcattgccatactgctggacgcccaccataagacctacgaccccacctactccgacttctgccagttccggcctccagttcgtgtgaatgatggtggagggagccatccttccaggcccaactccagacacactcccagcttctctggggactcctcctcctcctgctcagatcactgtatcacctcttcagacatgatggactcgtccagcttctccaatctggatctgagtgaagaagattcagatgacccttctgtgaccctagagctgtcccagctctccatgctgccccacctggctgacctggtcagttacagcatccaaaaggtcattggctttgctaagatgataccaggattcagagacctcacctctgaggaccagatcgtactgctgaagtcaagtgccattgaggtcatcatgttgcgctccaatgagtccttcaccatggacgacatgtcctggacctgtggcaaccaagactacaagtaccgcgtcagtgacgtgaccaaagccggacacagcctggagctgattgagcccctcatcaagttccaggtgggactgaagaagctgaacttgcatgaggaggagcatgtcctgctcatggccatctgcatcgtctccccagatcgtcctggggtgcaggacgccgcgctgattgaggccatccaggaccgcctgtccaacacactgcagacgtacatccgctgccgccacccgcccccgggcagccacctgctctatgccaagatgatccagaagctagccgacctgcgcagcctcaatgaggagcactccaagcagtaccgctgcctctccttccagcctgagtgcagcatgaagctaacgccccttgtgctcgaagtgtttggcaatgagatctcctgactaggacagcctgtggcggtgcctgggtggggctgctcctccagggccacgtgccaggcccggggctggcggctactcagcagccctcctcaccccgtctggggttcagcccctcctctgccacctcccctatccacccagcccattctctctcctgtccaacctaacccctttcctgcgggcttttccccggtcccttgagacctcagccatgaggagttgctgtttgtttgacaaagaaacccaagtgggggcagagggcagaggctggaggcagggccttgcccagagatgcctccaccgctgcctaagtggctgctgactgatgttgagggaacagacaggagaaatgcatccattcctcagggacagagacacctgcacctccccccactgcaggccccgcttgtccagcgcctagtggggtctccctctcctgcctactcacgataaataatcggcccacagctcccaccccacccccttcagtgcccaccaacatcccattgccctggttatattctcacgggcagtagctgtggtgaggtgggttttcttcccatcactggagcaccaggcacgaacccacctgctgagagacccaaggaggaaaaacagacaaaaacagcctcacagaagaatatgacagctgtccctgtcaccaagctcacagttcctcgccctgggtctaaggggttggttgaggtggaagccctccttccacggatccatgtagcaggactgaattgtccccagtttgcagaaaagcacctgccgacctcgtcctccccctgccagtgccttacctcctgcccaggagagccagccctccctgtcctcctcggatcaccgagagtagccgagagcctgctcccccaccccctccccaggggagagggtctggagaagcagtgagccgcatcttctccatctggcagggtgggatggaggagaagaattttcagaccccagcggctgagtcatgatctccctgccgcctcaatgtggttgcaaggccgctgttcacccacagggctaagagctagcgctgccgcaccccagagtgtgggaagggagagcggggcagtctcgggtggctagtcagagagagtgtttgggggttccgtgatgtagggtaaggtgccttcttattctcactccaccacccaaaagtcaaaaggtgcctgtgaggcaggggcggagtgatacaacttcaagtgcatgctctctgcagccagcccagcccagctggtgggaagcgtctgtccgtttactccaaggtggggtctttgtgagagtgagctgtaggtgtgcgggaccggtacagaaaggcgttcttcgaggtggatcacagaggcttcttcagatcagtgcttgagtttggggaatgcggccgcattccctgagtcaccaggaatgttaaagtcagtgggaacgtgactgccccaactcctggaagctgtgtccttgcacctgcatccgtagttccctgaaaacccagagaggaatcagacttcacactgcaagagccttggtgtccacctggccccatgtctctcagaattcttcaggtggaaaaacatctgaaagccacgttccttactgcagaatagcatatatatcgcttaatcttaaatttattagatatgagttgttttcagactcagactccatttgtattatagtctaatatacagggtagcaggtaccactgatttggagatatttatggggggagaacttacattgtgaaacttctgtacattaattattattgctgttgttattttacaagggtctagggagagacccttgtttgattttagctgcagaacgtattggtccagcttgctcttcagtgggagaaaacacttgtaagttgctaaacgagtcaatcccctcattcaggaaaactgacagaggagggcgtgactcacccaagcatatataactagctagaagtgggccaggacaggcccggcgcggtggctcacgcctgtaatcccagcagtttgggaggtcgaggtaggtggatcacctgaggtcgggagttcgagaccaacctgaccaacatggagaaaccctgtctctattaaaaatacaaaaaaaaaaaaaaaaaaaatagccgggcatggtggcgcaagcctgtaatcccagctactcaggaggctgaggcagaagaattgaacccaggaggtggaggttgcagtgagctgagatcgtgccgttactctccaacctggacaacaagagcgaaactccgtcttagaagtggaccaggacaggaccagattttggagtcatggtccggtgtccttttcactacaccatgtttgagctcagacccccactctcattccccaggtggctgacccagtccctgggggaagccctggatttcagaaagagcaagtctggatctgggaccctttccttccttccctggcttgtaactccaccaacccatcagaaggagaaggaaggagactcacctctgcctcaatgtgaatcagaccctaccccaccacgatgtggccctggcctgctgggctctccacctcagccttggataatgctgttgcctcatctataacatgcatttgtctttgtaatgtcaccaccttcccagctctccctctggccctgccttcttcggggaactcctggaaatatcagttactcagccctgggccccaccacctaggccactcctccaaaggaagtctaggagctgggaggaaaagaaaagaggggaaaatgagtttttatggggctgaacggggagaaaaggtcatcatcgattctactttagaatgagagtgtgaaatagacatttgtaaatgtaaaacttttaaggtatatcattataactgaaggagaaggtgccccaaaatgcaagattttccacaagattcccagagacaggaaaatcctctggctggctaactggaagcatgtaggagaatccaagcgaggtcaacagagaaggcaggaatgtgtggcagatttagtgaaagctagagatatggcagcgaaaggatgtaaacagtgcctgctgaatgatttccaaagagaaaaaaagtttgccagaagtttgtcaagtcaaccaatgtagaaagctttgcttatggtaataaaaatggctcatacttatatagcacttactttgttgcaagtactgctgtaaataaatgctttatgcaaaccaa